European Patent Specification EP 3 316 909 B1, published August 30, 2023. Title: ANTI-NTB-A ANTIBODIES AND RELATED COMPOSITIONS AND METHODS. Applicant: SEATTLE GENETICS, INC. The sequence listing filed with the application follows.

SEQUENCE LISTING (29 sequences)

SEQ ID NO: 1 - protein, 332 aa, Homo sapiens
MLWLFQSLLFVFCFGPGNVVSQSSLTPLMVNGILGESVTLPLEFPAGEKVNFITWLFNETSLAFIVPHETKSPEIHVTNPKQGKRLNFTQSYSLQLSNLKMEDTGSYRAQISTKTSAKLSSYTLRILRQLRNIQVTNHSQLFQNMTCELHLTCSVEDADDNVSFRWEALGNTLSSQPNLTVSWDPRISSEQDYTCIAENAVSNLSFSVSAQKLCEDVKIQYTDTKMILFMVSGICIVFGFIILLLLVLRKRRDSLSLSTQRTQGPAESARNLEYVSVSPTNNTVYASVTHSNRETEIWTPRENDTITIYSTINHSKESKPTFSRATALDNVV

SEQ ID NO: 2 - protein, 332 aa, Macaca fascicularis
MLWLFQSLLFVFCFGPGNLVSQSSSTPLMVNGVLGESVILPLELSAGEMIASITWLCNGTSLAFIEPSETKSPNIRVTHPKQRKRLNFTQSYSLKLSNLEMEDTGSYSAQITTETSVKLSSYTLRIFRQLRSIQVNNYSQLFQNRTCEIHLTCSVEDADDNVSFRWEALGSTLSSEPNITTSWDPRISGEQDYTCIAENAVSNLSFSVSAQKLCGDVKIQYTDTKMILFVVFGICIVTGFIIMLLLVLRKRRDSLPLSTQRTQGPAEPAGNIEYVSVSPVNNTVYASVTHSNRETEISTPIKNATVTIYSTVNHSKESKPTFSRATALDNVV

SEQ ID NO: 3 - protein, 118 aa, Mus musculus
QIQLVQSGPELKKPGETVKISCKASGYTFTNYGMNWVKQAPGKDLKWMGWINTYSGEPRYADDFKGRFAFSLEKSANTAYLQINNLKNEDMATYFCARDYGRWYFDVWGTGTTVTVSS

SEQ ID NO: 4 - protein, 118 aa, Artificial
  mature heavy chain variable region of humanized 20F3 with no back mutations
QVQLVQSGSELKKPGASVKVSCKASGYTFTNYGMNWVRQAPGQGLEWMGWINTYSGEPRYADDFKGRFVFSLDTSVSTAYLQISSLKAEDTAVYYCARDYGRWYFDVWGQGTTVTVSS

SEQ ID NO: 5 - protein, 118 aa, Artificial; identical to SEQ ID NO: 4
  mature heavy chain variable region of humanized 20F3 HA

SEQ ID NO: 6 - protein, 118 aa, Artificial
  mature heavy chain variable region of humanized 20F3 HB
QIQLVQSGSELKKPGASVKVSCKASGYTFTNYGMNWVRQAPGQGLEWMGWINTYSGEPRYADDFKGRFVFSLDKSVSTAYLQISSLKAEDTAVYYCARDYGRWYFDVWGQGTTVTVSS

SEQ ID NO: 7 - protein, 118 aa, Artificial
  mature heavy chain variable region of humanized 20F3 HC
QIQLVQSGSELKKPGASVKVSCKASGYTFTNYGMNWVRQAPGQDLEWMGWINTYSGEPRYADDFKGRFVFSLDKSVNTAYLQISSLKAEDTAVYYCARDYGRWYFDVWGQGTTVTVSS

SEQ ID NO: 8 - protein, 118 aa, Artificial
  mature heavy chain variable region of humanized 20F3 HD
QIQLVQSGSELKKPGASVKVSCKASGYTFTNYGMNWVRQAPGQDLKWMGWINTYSGEPRYADDFKGRFVFSLDKSVNTAYLQISSLKAEDTAVYYCARDYGRWYFDVWGQGTTVTVSS

SEQ ID NO: 9 - protein, 118 aa, Artificial
  mature heavy chain variable region of humanized 20F3 HE
QIQLVQSGSELKKPGASVKVSCKASGYTFTNYGMNWVKQAPGQDLKWMGWINTYSGEPRYADDFKGRFAFSLDKSVNTAYLQISSLKAEDTAVYFCARDYGRWYFDVWGQGTTVTVSS

SEQ ID NO: 10 - protein, 5 aa, Mus musculus
NYGMN

SEQ ID NO: 11 - protein, 17 aa, Mus musculus
WINTYSGEPRYADDFKG

SEQ ID NO: 12 - protein, 9 aa, Mus musculus
DYGRWYFDV

SEQ ID NO: 13 - protein, 107 aa, Mus musculus
QIVLSQSPAILSASPGEKVTMTCRASSSVSHMHWYQQKPGSSPKPWIYATSNLASGVPARFSGSGSGTSYSLTISRVEAEDAATYYCQQWSSTPRTFGGGTKLEIKR

SEQ ID NO: 14 - protein, 107 aa, Artificial
  mature light chain variable region of humanized 20F3 with no back mutations
EIVLTQSPATLSLSPGERATLSCRASSSVSHMHWYQQKPGQAPRLLIYATSNLASGIPARFSGSGSGTDFTLTISSLEPEDFAVYYCQQWSSTPRTFGGGTKVEIKR

SEQ ID NO: 15 - protein, 107 aa, Artificial; identical to SEQ ID NO: 14
  mature light chain variable region of humanized 20F3 LA

SEQ ID NO: 16 - protein, 107 aa, Artificial
  mature light chain variable region of humanized 20F3 LB
EIVLTQSPATLSLSPGERATLSCRASSSVSHMHWYQQKPGQAPRPWIYATSNLASGIPARFSGSGSGTDYTLTISSLEPEDFAVYYCQQWSSTPRTFGGGTKVEIKR

SEQ ID NO: 17 - protein, 107 aa, Artificial
  mature light chain variable region of humanized 20F3 LC
QIVLSQSPATLSLSPGERATLSCRASSSVSHMHWYQQKPGQAPRPWIYATSNLASGIPARFSGSGSGTDYTLTISSLEPEDFAVYYCQQWSSTPRTFGGGTKVEIKR

SEQ ID NO: 18 - protein, 107 aa, Artificial
  mature light chain variable region of humanized 20F3 LD
QIVLSQSPATLSLSPGERATMSCRASSSVSHMHWYQQKPGQAPRPWIYATSNLASGVPARFSGSGSGTDYTLTISSLEPEDFAVYYCQQWSSTPRTFGGGTKVEIKR

SEQ ID NO: 19 - protein, 10 aa, Mus musculus
RASSSVSHMH

SEQ ID NO: 20 - protein, 7 aa, Mus musculus
ATSNLAS

SEQ ID NO: 21 - protein, 9 aa, Mus musculus
QQWSSTPRT

SEQ ID NO: 22 - protein, 8 aa, Mus musculus
GYTFTNYG

SEQ ID NO: 23 - protein, 8 aa, Mus musculus
INTYSGEP

SEQ ID NO: 24 - protein, 11 aa, Mus musculus
ARDYGRWYFDV

SEQ ID NO: 25 - protein, 5 aa, Mus musculus
SSVSH

SEQ ID NO: 26 - protein, 9 aa, Mus musculus
QQWSSTPRT

SEQ ID NO: 27 - protein, 106 aa, Homo sapiens
TVAAPSVFIFPPSDEQLKSGTASVVCLLNNFYPREAKVQWKVDNALQSGNSQESVTEQDSKDSTYSLSSTLTLSKADYEKHKVYACEVTHQGLSSPVTKSFNRGEC

SEQ ID NO: 28 - protein, 329 aa, Homo sapiens
ASTKGPSVFPLAPSSKSTSGGTAALGCLVKDYFPEPVTVSWNSGALTSGVHTFPAVLQSSGLYSLSSVVTVPSSSLGTQTYICNVNHKPSNTKVDKKVEPKSCDKTHTCPPCPAPELLGGPSVFLFPPKPKDTLMISRTPEVTCVVVDVSHEDPEVKFNWYVDGVEVHNAKTKPREEQYNSTYRVVSVLTVLHQDWLNGKEYKCKVSNKALPAPIEKTISKAKGQPREPQVYTLPPSRDELTKNQVSLTCLVKGFYPSDIAVEWESNGQPENNYKTTPPVLDSDGSFFLYSKLTVDKSRWQQGNVFSCSVMHEALHNHYTQKSLSLSPG

SEQ ID NO: 29 - protein, 329 aa, Artificial
  variant heavy chain constant region (S239C)
ASTKGPSVFPLAPSSKSTSGGTAALGCLVKDYFPEPVTVSWNSGALTSGVHTFPAVLQSSGLYSLSSVVTVPSSSLGTQTYICNVNHKPSNTKVDKKVEPKSCDKTHTCPPCPAPELLGGPCVFLFPPKPKDTLMISRTPEVTCVVVDVSHEDPEVKFNWYVDGVEVHNAKTKPREEQYNSTYRVVSVLTVLHQDWLNGKEYKCKVSNKALPAPIEKTISKAKGQPREPQVYTLPPSRDELTKNQVSLTCLVKGFYPSDIAVEWESNGQPENNYKTTPPVLDSDGSFFLYSKLTVDKSRWQQGNVFSCSVMHEALHNHYTQKSLSLSPG